European Patent Specification EP 3 334 709 B1, published December 11, 2024. Title: SALTS OF AN LSD1 INHIBITOR. Applicant: Incyte Corporation LI, Qun. The sequence listing filed with the application follows.

SEQUENCE LISTING (1 sequence)

SEQ ID NO: 1 - protein, 24 aa, Artificial Sequence
  synthetic peptide
  INIT_MET (4)..(4)
ARTKQTARKSTGGKAPRKQLAGGK